European Patent Specification EP 4 037 481 B1, published September 11, 2024. Title: A CRNN LOSS OF FUNCTION RODENT MODEL. Applicant: Regeneron Pharmaceuticals, Inc. The sequence listing filed with the application follows.

SEQUENCE LISTING (6 sequences)

SEQ ID NO: 1 - DNA, 1902 bp, Homo sapiens
actcctcacaccacttaacagccacttgtttcatcccacctgggcattaggttgacttcaaagatgcctcagttactgcaaaacattaatgggatcatcgaggccttcaggcgctatgcaaggacggagggcaactgcacagcgctcacccgaggggagctgaaaagactcttggagcaagagtttgccgatgtgattgtgaaaccccacgatccagcaactgtggatgaggtcctgcgtctgctggatgaagaccacacagggactgtggaattcaaggaattcctggtcttagtgtttaaagttgcccaggcctgtttcaagacactgagcgagagtgctgagggagcctgcggctctcaagagtctggaagcctccactctggggcctcgcaggagctgggcgaaggacagagaagtggcactgaagtgggaagggcggggaaagggcagcattatgaggggagcagccacagacagagccagcagggttccagagggcagaacaggcctggggttcagacccagggtcaggccactggctctgcgtgggtcagcagctatgacaggcaagctgagtcccagagccaggaaagaataagcccgcagatacaactctctgggcagacagagcagacccagaaagctggagaaggcaagaggaatcagacaacagagatgaggccagagagacagccacagaccagggaacaggacagagcccaccagacaggtgagactgtgactggatctggaactcagacccaggcaggtgccacccagactgtggagcaggacagcagccaccagacaggaagaaccagcaagcagacacaggaggccaccaatgaccagaacagagggactgagacccacggtcaaggcaggagccagaccagccaggctgtgacaggaggacatgctcagatacaggcagggacacacacccagacacccacccagaccgtggagcaggacagcagccaccagacaggaagcaccagcacccagacacaggagtccaccaatggccagaacagagggactgagatccacggtcaaggcaggagccagaccagccaggctgtgacaggaggacacactcagatacaggcagggtcacacaccgagactgtggagcaggacagaagccaaactgtaagccacggaggggctagagaacagggacagacccagacgcagccaggcagtggtcaaagatggatgcaagtgagcaaccctgaggcaggagagacagtaccgggaggacaggcccagactggggcaagcactgagtcaggaaggcaggagtggagcagcactcacccaaggcgctgtgtgacagaagggcagggagacagacagcccacagtggttggtgaggaatgggttgatgaccactcaagggagacagtgatcctcaggctggaccagggcaacttgcataccagtgtttcctcagcacagggccaggatgcagcccagtcagaagagaagcgaggcatcacagctagagagctgtattcctacttgagaagcaccaagccatgacttccccgactccaatgtccagtactggaagaagacagctggagagagtttggcttgtcctgcatggccaatccagtgggtgcatccctggacatcagctcttcattatgcagcttcccttttaggtctttctcaatgagataatttctgcaaggagctttctatcctgaactcttctttcttacctgctttgcggtgcagaccctctcaggagcaggaagactcagagcaagtcacccctttgtactgaattgtcctcatcttgtggggggtttcaggactatttttatctctgacatctctctattgccccatctaccctaatgcatcaataaaaccttaagccactgg

SEQ ID NO: 2 - protein, 495 aa, Homo sapiens
MPQLLQNINGIIEAFRRYARTEGNCTALTRGELKRLLEQEFADVIVKPHDPATVDEVLRLLDEDHTGTVEFKEFLVLVFKVAQACFKTLSESAEGACGSQESGSLHSGASQELGEGQRSGTEVGRAGKGQHYEGSSHRQSQQGSRGQNRPGVQTQGQATGSAWVSSYDRQAESQSQERISPQIQLSGQTEQTQKAGEGKRNQTTEMRPERQPQTREQDRAHQTGETVTGSGTQTQAGATQTVEQDSSHQTGRTSKQTQEATNDQNRGTETHGQGRSQTSQAVTGGHAQIQAGTHTQTPTQTVEQDSSHQTGSTSTQTQESTNGQNRGTEIHGQGRSQTSQAVTGGHTQIQAGSHTETVEQDRSQTVSHGGAREQGQTQTQPGSGQRWMQVSNPEAGETVPGGQAQTGASTESGRQEWSSTHPRRCVTEGQGDRQPTVVGEEWVDDHSRETVILRLDQGNLHTSVSSAQGQDAAQSEEKRGITARELYSYLRSTKP

SEQ ID NO: 3 - DNA, 1973 bp, Mus musculus
actctacacactgcttaacagaaacttgtcccatcctgcctgagcattagcatagcttcaaagatgcctcagttgctgcaaaacatccacgggatcatcgaagccttcgggtgctatgccaggtcagagggtggctgcaaagtactcacgaggcaggagttgaagaggctcctggaacatgagtttgctgacgtcatagtgaagccccatgatcctgcaactgtggatgaagtcctgcgcctgttggatgaagataacacagggactgtagagttcaaggaattcctagtcttggtgtttaaagttgcacgggcttgctttaagacactgaatgagagtcctaagggtgcttgcatatctgacaagtctgaaggctgctattctggatcttcaaaagagctggagcaaagacagagaggtggtgctgaagtggcaaaagacggagcagcacagcactgtgaagacagcagctgtggacagagagatcaggcttctagaggacaggacagggttgggacacatacccagaatcaggacagctaccctacacaggtcagcagtcatgacaggcagactgagtctcagacacaggaaatgataagccaacaaacacaagtgacaggacaggtggagcagaccccaagaacagaagacaagagttggaccagacagaagaggtcagagaggcaaccacagagtagccaacagacagatgagatcacaactggatctacagctcagacccaagcaggtaacttctacacacaggggtctacctgtgactataacagaggaactaacagccatcaccaagacagaagccatgcagacagagcttctacacaacactaccagacacaggcagggtctcatactcagatacacacacagatggtagaacaggcctgggggcagcaaacaggaagtgatagcatccagacacaggggtctatctatgaccagagcactgagactgtgattcatggccaagacaggaaccaggcaagccagagtgttaaagaacaccaccaggcacagggagagtcatatattcagacacatactcagacaatggaacaaggcaggagccagcaggcagaaaatagtagcacccagactcatgggtccatgtatggccaaaacagagagactgagatccatgggctagaaagcagtcaggcagaacaggtggggacaagacactaccagacacaggcaggatcatatacccagactttggaacatgatgggagccagtctgcacataaatttgtggctcaagaaaaggaacgtacacagacaaagccatgcatggggcaaagctggacaccagtaagcaactatgagacagaagagtcagtgataggaggacaggtccagactgagacagacactattatagagaatcacccaagcccgacagccaggcaggtagagagagtacccacagtggttagagaggagtgggtcaatgaccacacaagggaaatagtaatccgaagccaggatccaggtagcctgcactctggtactccttcagctcagggccaggatataccacagatggagaagaaaggaatcacagccaagggactatatacctacttgaagacagagcagccatgacttttcccgattccagctggagtgaggttggcctgccctgccctgccctgccctgccctgccctgccctgccctgccctgccctgccatggtacttcaccagacagccatgattcttcttgtttggttcttttacagtgatcatctctacaaggtgatttcttgtcaaaactcacctctcttacctgctgctctcagaaactcacctctcttacctgatattctcagaaacaggaagatgtggaggaggtcatctcattgcactgaattccccccaattttcagggggtttcaaagctgttttatctctggtatctgtccattgcatcaataaaggcttagaagctg

SEQ ID NO: 4 - protein, 520 aa, Mus musculus
MPQLLQNIHGIIEAFGCYARSEGGCKVLTRQELKRLLEHEFADVIVKPHDPATVDEVLRLLDEDNTGTVEFKEFLVLVFKVARACFKTLNESPKGACISDKSEGCYSGSSKELEQRQRGGAEVAKDGAAQHCEDSSCGQRDQASRGQDRVGTHTQNQDSYPTQVSSHDRQTESQTQEMISQQTQVTGQVEQTPRTEDKSWTRQKRSERQPQSSQQTDEITTGSTAQTQAGNFYTQGSTCDYNRGTNSHHQDRSHADRASTQHYQTQAGSHTQIHTQMVEQAWGQQTGSDSIQTQGSIYDQSTETVIHGQDRNQASQSVKEHHQAQGESYIQTHTQTMEQGRSQQAENSSTQTHGSMYGQNRETEIHGLESSQAEQVGTRHYQTQAGSYTQTLEHDGSQSAHKFVAQEKERTQTKPCMGQSWTPVSNYETEESVIGGQVQTETDTIIENHPSPTARQVERVPTVVREEWVNDHTREIVIRSQDPGSLHSGTPSAQGQDIPQMEKKGITAKGLYTYLKTEQP

SEQ ID NO: 5 - DNA, 2551 bp, Rattus norvegicus
tgatgacacttaatagctaccacttagcataagccaagcatcagctgggtgctttttatgaattatctcctaaagcctttatgatacctctctgaagtaagtgctagtatcagctccattcacagtgaagaaactgaggcatggacaagcaaagcaggtaggtggtggaacccggcattaaatgttgactcagaaatttccatggtctgagtgactctccttcccatcataaagtacattttgaggagaagaacaaggaaggtggagaaacccaaacacagctgaagacacaatgaaaggaccgggccttggcatactgtgtggaaacatcaggggctgactatggtgcccataaaaagcattttcatattttccagcatagcttcaaagatgcctcagttgctgcgaaatatccatgggatcatcgaagccttcgggtgctatgccaggtcagagggtggctgcaaagtactcacgaagcaggagctgaagaggcttctggaatatgagtttgccgacgtcatagtgaagccccatgatcctgcaactgtggatgaagttctgcacctgttggatgaagataacacaggaactgtagaattcaaggaattcttggtcttggtgtttaaagttgcccgtgcctgctttaagacactgaatgagagtcctaagggtgcttgcatgtctgacaagtctgaaagctgccatgttggatcttccaaagagctggagcaaggacagaggggtggtgctgaagtggcaaaggatggagcagcacagcactgtgaaaacagcagttgtggacagagagatcaggcttctagaggacaggacagggtggggacacatacccagcatcaggacagctaccctacatgggtcagcagtcatgacaggcaggctgagtctcagacacaggagatgataagccagcaaacacaagtgacaggaccagtggaacagaccccaaaaatagaagacaagagttgcatcggacagaagagatcagagagacaaccacagatcagccaacagacagatgagatcacaactgaatccacaactcagacccaagcaggcaccttctacacacagggatctacctgtgatcagaacagaggaacaaacagccttacccaagacagaagtcagacagaccaagcttctacacaacactaccagacacgggcagggtctcatactcagatacacaaccagacggtggaacagggctggggacagcagacaggaaaaaacaacatccaaatacagggatctatctatgaccagagcagagagactgagattcgtggccaagataggaaccaggcaagccagactgctaaagaacaccaccaggcacaggcagagtcatatactcgggcgcacactcagacaatggaacaaggcaggagccagcaggaagaaaatggcagtatccagactcatgcttccatctgtggccaaaacagaggaaccaagatccatgagcaagaaagcaatcaggtagaacaggtgggaacaggacactgccagacacaggcaggatcagatgcccagactttggagcataatgggagccattctgcacgacaagtagtggctcaagaaaagggacaaatgcagacacagtcatgcatggggcaaagctggacaccagtgagcaactatgagacaggagagccagtgctaggacaggtccagactgagatagacactgttaaagaaagacaaccgtggaacagcaatcacccaagtctggcaggaaggcagggagaaagaagccccacagtggttagagaggagtgggtcaatgaccacacaagagaaatagtgatccgaagccaggatccaggcagcctgcactctggtgctccttcagctcagggccaggatacagcacagatggagaagaaaggaatcacagccaagggattatattcgtacctgaagacagagcagccatgacttctcctgactccagtgcccataccaaaagacagctgcagtgaggttggcctgccttgtcctgtgctgccctgtcacagcacttcactggacagctatgattcttctcatttggttctttttcagcaatcatttctacaaggtgatttcttgtctaaacttacctctcttgcccggtgctctcagaaactcacctctcttatctgctactctcaggaacaggaagccatggaggaggtcatctcattgcactgaatttcttccaactttcagggggtttcaaagctgttttatctctgctatcggtccattgcatcaataaaggcttagcagctggtttcagtgtgttattcaatagtttctactgatgtgacaaactgagagctctagagttctgatgttgaactgaacatagcctcatctctcaaggaagactgagttagaacgagctaaatagaggagagagcacactgtatacttggcagagatgggtcagggatgtcttcttccataaagatgcttatttgtagtagccctcaaaaggacaactaagagaaacagagatataattactatcattcag

SEQ ID NO: 6 - protein, 541 aa, Rattus norvegicus
MVPIKSIFIFSSIASKMPQLLRNIHGIIEAFGCYARSEGGCKVLTKQELKRLLEYEFADVIVKPHDPATVDEVLHLLDEDNTGTVEFKEFLVLVFKVARACFKTLNESPKGACMSDKSESCHVGSSKELEQGQRGGAEVAKDGAAQHCENSSCGQRDQASRGQDRVGTHTQHQDSYPTWVSSHDRQAESQTQEMISQQTQVTGPVEQTPKIEDKSCIGQKRSERQPQISQQTDEITTESTTQTQAGTFYTQGSTCDQNRGTNSLTQDRSQTDQASTQHYQTRAGSHTQIHNQTVEQGWGQQTGKNNIQIQGSIYDQSRETEIRGQDRNQASQTAKEHHQAQAESYTRAHTQTMEQGRSQQEENGSIQTHASICGQNRGTKIHEQESNQVEQVGTGHCQTQAGSDAQTLEHNGSHSARQVVAQEKGQMQTQSCMGQSWTPVSNYETGEPVLGQVQTEIDTVKERQPWNSNHPSLAGRQGERSPTVVREEWVNDHTREIVIRSQDPGSLHSGAPSAQGQDTAQMEKKGITAKGLYSYLKTEQP